European Patent Application EP 4 793 288 A1, published August 19, 2026. Title: HLA-G에 특이적으로 결합하는 항체 및 이의 용도. Applicant: 주식회사 아이엠바이오로직스. The sequence listing filed with the application follows.

SEQUENCE LISTING (223 sequences)

SEQ ID NO: 1 - protein, 5 aa, synthetic construct
SYAMS

SEQ ID NO: 2 - protein, 17 aa, synthetic construct
RISGSGGYIYYADSVKG

SEQ ID NO: 3 - protein, 12 aa, synthetic construct
EGTSSYRGWMDV

SEQ ID NO: 4 - protein, 11 aa, synthetic construct
RASQSISNYLN

SEQ ID NO: 5 - protein, 7 aa, synthetic construct
AASSLQS

SEQ ID NO: 6 - protein, 10 aa, synthetic construct
CQQSYSSPWT

SEQ ID NO: 7 - protein, 30 aa, synthetic construct
EVQLVESGGGLVQPGGSLRLSCAASGFTFS

SEQ ID NO: 8 - protein, 14 aa, synthetic construct
WVRQAPGKGLEWVS

SEQ ID NO: 9 - protein, 32 aa, synthetic construct
RFTISRDNSKNTLYLQMNSLRAEDTAVYYCAK

SEQ ID NO: 10 - protein, 11 aa, synthetic construct
WGQGTLVTVSS

SEQ ID NO: 11 - protein, 23 aa, synthetic construct
DIQMTQSPSSLSASVGDRVTITC

SEQ ID NO: 12 - protein, 15 aa, synthetic construct
WYQQKPGKAPKLLIY

SEQ ID NO: 13 - protein, 31 aa, synthetic construct
GVPSRFSGSGSGTDFTLTISSLQPEDFATYY

SEQ ID NO: 14 - protein, 10 aa, synthetic construct
FGQGTKVEIK

SEQ ID NO: 15 - protein, 121 aa, synthetic construct
EVQLVESGGGLVQPGGSLRLSCAASGFTFSSYAMSWVRQAPGKGLEWVSRISGSGGYIYYADSVKGRFTISRDNSKNTLYLQMNSLRAEDTAVYYCAKEGTSSYRGWMDVWGQGTLVTVSS

SEQ ID NO: 16 - protein, 107 aa, synthetic construct
DIQMTQSPSSLSASVGDRVTITCRASQSISNYLNWYQQKPGKAPKLLIYAASSLQSGVPSRFSGSGSGTDFTLTISSLQPEDFATYYCQQSYSSPWTFGQGTKVEIK

SEQ ID NO: 17 - protein, 5 aa, synthetic construct
SYAMS

SEQ ID NO: 18 - protein, 17 aa, synthetic construct
SISGSGNSELYAGSVKG

SEQ ID NO: 19 - protein, 14 aa, synthetic construct
FSAAVGFLPDYFDS

SEQ ID NO: 20 - protein, 11 aa, synthetic construct
QASHDISKYLN

SEQ ID NO: 21 - protein, 7 aa, synthetic construct
DASNLET

SEQ ID NO: 22 - protein, 9 aa, synthetic construct
QQSYRTPLT

SEQ ID NO: 23 - protein, 30 aa, synthetic construct
EVQLVESGGNWVQPGGSLRLSCAASGFSFR

SEQ ID NO: 24 - protein, 14 aa, synthetic construct
WVRQAPGKGLEWVS

SEQ ID NO: 25 - protein, 32 aa, synthetic construct
RFTISRDNSKNTLSLQLHSLRAEDTAMYYCAK

SEQ ID NO: 26 - protein, 11 aa, synthetic construct
WGQGTLVTVSS

SEQ ID NO: 27 - protein, 23 aa, synthetic construct
ELTLTQSPSSLSASVGDRVTITC

SEQ ID NO: 28 - protein, 15 aa, synthetic construct
WYQQKSGKAPKLLIY

SEQ ID NO: 29 - protein, 32 aa, synthetic construct
GVPSRFSGSGSGTDFTLTISSLQPEDFATYYC

SEQ ID NO: 30 - protein, 10 aa, synthetic construct
FGGGTKLEIK

SEQ ID NO: 31 - protein, 123 aa, synthetic construct
EVQLVESGGNWVQPGGSLRLSCAASGFSFRSYAMSWVRQAPGKGLEWVSSISGSGNSELYAGSVKGRFTISRDNSKNTLSLQLHSLRAEDTAMYYCAKFSAAVGFLPDYFDSWGQGTLVTVSS

SEQ ID NO: 32 - protein, 107 aa, synthetic construct
ELTLTQSPSSLSASVGDRVTITCQASHDISKYLNWYQQKSGKAPKLLIYDASNLETGVPSRFSGSGSGTDFTLTISSLQPEDFATYYCQQSYRTPLTFGGGTKLEIK

SEQ ID NO: 33 - protein, 7 aa, synthetic construct
RSSHYWG

SEQ ID NO: 34 - protein, 16 aa, synthetic construct
SIYYSGITYYNPSLKS

SEQ ID NO: 35 - protein, 18 aa, synthetic construct
HGSYDSWAGRYKWDRFDP

SEQ ID NO: 36 - protein, 11 aa, synthetic construct
QASHDISKYLN

SEQ ID NO: 37 - protein, 8 aa, synthetic construct
DASNLETG

SEQ ID NO: 38 - protein, 9 aa, synthetic construct
QQSYSTPLT

SEQ ID NO: 39 - protein, 30 aa, synthetic construct
QVQLQESGPGLVKPSETLSLTCTVSGGSID

SEQ ID NO: 40 - protein, 14 aa, synthetic construct
WIRQPPGKGLEWLG

SEQ ID NO: 41 - protein, 32 aa, synthetic construct
RVTISVDTSRNQFSLTLSSVTAADTAVYYCAR

SEQ ID NO: 42 - protein, 11 aa, synthetic construct
WGQGTPVTVSS

SEQ ID NO: 43 - protein, 23 aa, synthetic construct
ELQMTQSPSSLSASVGDRVTITC

SEQ ID NO: 44 - protein, 15 aa, synthetic construct
WYQQKSGKAPKLLIY

SEQ ID NO: 45 - protein, 31 aa, synthetic construct
VPSRFSGSGSGTDFTLTISSLQPEDFATYYC

SEQ ID NO: 46 - protein, 10 aa, synthetic construct
FGGGTKVEIK

SEQ ID NO: 47 - protein, 128 aa, synthetic construct
QVQLQESGPGLVKPSETLSLTCTVSGGSIDRSSHYWGWIRQPPGKGLEWLGSIYYSGITYYNPSLKSRVTISVDTSRNQFSLTLSSVTAADTAVYYCARHGSYDSWAGRYKWDRFDPWGQGTPVTVSS

SEQ ID NO: 48 - protein, 107 aa, synthetic construct
ELQMTQSPSSLSASVGDRVTITCQASHDISKYLNWYQQKSGKAPKLLIYDASNLETGVPSRFSGSGSGTDFTLTISSLQPEDFATYYCQQSYSTPLTFGGGTKVEIK

SEQ ID NO: 49 - protein, 5 aa, synthetic construct
SYAMS

SEQ ID NO: 50 - protein, 17 aa, synthetic construct
RISGSGGYIYYADSVKG

SEQ ID NO: 51 - protein, 12 aa, synthetic construct
EGTSSYRGWMDV

SEQ ID NO: 52 - protein, 11 aa, synthetic construct
RASQSISNYLN

SEQ ID NO: 53 - protein, 7 aa, synthetic construct
AASRLQS

SEQ ID NO: 54 - protein, 9 aa, synthetic construct
QQSYSTPWT

SEQ ID NO: 55 - protein, 30 aa, synthetic construct; identical to SEQ ID NO: 7

SEQ ID NO: 56 - protein, 14 aa, synthetic construct
WVRQAPGKGLEWVS

SEQ ID NO: 57 - protein, 32 aa, synthetic construct; identical to SEQ ID NO: 9

SEQ ID NO: 58 - protein, 11 aa, synthetic construct
WGQGTLVTVSS

SEQ ID NO: 59 - protein, 23 aa, synthetic construct
DIQMTQSPSSLSASVGDRVTITC

SEQ ID NO: 60 - protein, 15 aa, synthetic construct
WYQQKPGKAPKLLIY

SEQ ID NO: 61 - protein, 32 aa, synthetic construct
DVPSRFSGSGSGTDFTLTISSLQPEDFATYYC

SEQ ID NO: 62 - protein, 10 aa, synthetic construct
FGQGTKVEIK

SEQ ID NO: 63 - protein, 107 aa, synthetic construct
DIQMTQSPSSLSASVGDRVTITCRASQSISNYLNWYQQKPGKAPKLLIYAASRLQSDVPSRFSGSGSGTDFTLTISSLQPEDFATYYCQQSYSTPWTFGQGTKVEIK

SEQ ID NO: 64 - protein, 5 aa, synthetic construct
SYAMS

SEQ ID NO: 65 - protein, 17 aa, synthetic construct
RISGSGGYIYYADSVKG

SEQ ID NO: 66 - protein, 12 aa, synthetic construct
EGTSSYRGWMDV

SEQ ID NO: 67 - protein, 11 aa, synthetic construct
RASQSISNWLN

SEQ ID NO: 68 - protein, 7 aa, synthetic construct
AASRLQS

SEQ ID NO: 69 - protein, 9 aa, synthetic construct
QQSYTSPWT

SEQ ID NO: 70 - protein, 30 aa, synthetic construct; identical to SEQ ID NO: 7

SEQ ID NO: 71 - protein, 14 aa, synthetic construct
WVRQAPGKGLEWVS

SEQ ID NO: 72 - protein, 32 aa, synthetic construct; identical to SEQ ID NO: 9

SEQ ID NO: 73 - protein, 11 aa, synthetic construct
WGQGTLVTVSS

SEQ ID NO: 74 - protein, 23 aa, synthetic construct
DIQMTQSPSSLSASVGDRVTITC

SEQ ID NO: 75 - protein, 15 aa, synthetic construct
WYQQKPGKAPKLLIY

SEQ ID NO: 76 - protein, 32 aa, synthetic construct; identical to SEQ ID NO: 29

SEQ ID NO: 77 - protein, 10 aa, synthetic construct
FGQGTKVEIK

SEQ ID NO: 78 - protein, 107 aa, synthetic construct
DIQMTQSPSSLSASVGDRVTITCRASQSISNWLNWYQQKPGKAPKLLIYAASRLQSGVPSRFSGSGSGTDFTLTISSLQPEDFATYYCQQSYTSPWTFGQGTKVEIK

SEQ ID NO: 79 - protein, 5 aa, synthetic construct
SYAMS

SEQ ID NO: 80 - protein, 17 aa, synthetic construct
RISGSGGYIYYADSVKG

SEQ ID NO: 81 - protein, 12 aa, synthetic construct
EGTSSYRGWMDV

SEQ ID NO: 82 - protein, 11 aa, synthetic construct
RASQSISNYLN

SEQ ID NO: 83 - protein, 7 aa, synthetic construct
ATSRLQS

SEQ ID NO: 84 - protein, 10 aa, synthetic construct
CQQSYSFPWT

SEQ ID NO: 85 - protein, 30 aa, synthetic construct; identical to SEQ ID NO: 7

SEQ ID NO: 86 - protein, 14 aa, synthetic construct
WVRQAPGKGLEWVS

SEQ ID NO: 87 - protein, 32 aa, synthetic construct; identical to SEQ ID NO: 9

SEQ ID NO: 88 - protein, 11 aa, synthetic construct
WGQGTLVTVSS

SEQ ID NO: 89 - protein, 23 aa, synthetic construct
DIQMTQSPSSLSASVGDRVTITC

SEQ ID NO: 90 - protein, 15 aa, synthetic construct
WYQQKPGKAPKLLIY

SEQ ID NO: 91 - protein, 31 aa, synthetic construct; identical to SEQ ID NO: 13

SEQ ID NO: 92 - protein, 10 aa, synthetic construct
FGQGTKVEIK

SEQ ID NO: 93 - protein, 107 aa, synthetic construct
DIQMTQSPSSLSASVGDRVTITCRASQSISNYLNWYQQKPGKAPKLLIYATSRLQSGVPSRFSGSGSGTDFTLTISSLQPEDFATYYCQQSYSFPWTFGQGTKVEIK

SEQ ID NO: 94 - protein, 5 aa, synthetic construct
SYAMS

SEQ ID NO: 95 - protein, 17 aa, synthetic construct
RISGSGGYIYYADSVKG

SEQ ID NO: 96 - protein, 12 aa, synthetic construct
EGTSSYRGWMDV

SEQ ID NO: 97 - protein, 11 aa, synthetic construct
RASQSISRYLN

SEQ ID NO: 98 - protein, 7 aa, synthetic construct
ATSNLHS

SEQ ID NO: 99 - protein, 10 aa, synthetic construct
CQQSYTSPWT

SEQ ID NO: 100 - protein, 30 aa, synthetic construct; identical to SEQ ID NO: 7

SEQ ID NO: 101 - protein, 14 aa, synthetic construct
WVRQAPGKGLEWVS

SEQ ID NO: 102 - protein, 32 aa, synthetic construct; identical to SEQ ID NO: 9

SEQ ID NO: 103 - protein, 11 aa, synthetic construct
WGQGTLVTVSS

SEQ ID NO: 104 - protein, 23 aa, synthetic construct
DIQMTQSPSSLSASVGDRVTITC

SEQ ID NO: 105 - protein, 15 aa, synthetic construct
WYQQKPGKAPKLLIY

SEQ ID NO: 106 - protein, 31 aa, synthetic construct; identical to SEQ ID NO: 13

SEQ ID NO: 107 - protein, 10 aa, synthetic construct
FGQGTKVEIK

SEQ ID NO: 108 - protein, 107 aa, synthetic construct
DIQMTQSPSSLSASVGDRVTITCRASQSISRYLNWYQQKPGKAPKLLIYATSNLHSGVPSRFSGSGSGTDFTLTISSLQPEDFATYYCQQSYTSPWTFGQGTKVEIK

SEQ ID NO: 109 - protein, 5 aa, synthetic construct
DYAMS

SEQ ID NO: 110 - protein, 17 aa, synthetic construct
RISQSGSYTYYADSVKG

SEQ ID NO: 111 - protein, 12 aa, synthetic construct
EGTSSYRGWMDV

SEQ ID NO: 112 - protein, 11 aa, synthetic construct
RASQSISSYLN

SEQ ID NO: 113 - protein, 7 aa, synthetic construct
AASRLQS

SEQ ID NO: 114 - protein, 9 aa, synthetic construct
QQSYSTPWT

SEQ ID NO: 115 - protein, 30 aa, synthetic construct; identical to SEQ ID NO: 7

SEQ ID NO: 116 - protein, 14 aa, synthetic construct
WVRQAPGKGLEWVS

SEQ ID NO: 117 - protein, 32 aa, synthetic construct; identical to SEQ ID NO: 9

SEQ ID NO: 118 - protein, 11 aa, synthetic construct
WGQGTLVTVSS

SEQ ID NO: 119 - protein, 23 aa, synthetic construct
DIQMTQSPSSLSASVGDRVTITC

SEQ ID NO: 120 - protein, 15 aa, synthetic construct
WYQQKPGKAPKLLIY

SEQ ID NO: 121 - protein, 32 aa, synthetic construct; identical to SEQ ID NO: 29

SEQ ID NO: 122 - protein, 10 aa, synthetic construct
FGQGTKVEIK

SEQ ID NO: 123 - protein, 121 aa, synthetic construct
EVQLVESGGGLVQPGGSLRLSCAASGFTFSDYAMSWVRQAPGKGLEWVSRISQSGSYTYYADSVKGRFTISRDNSKNTLYLQMNSLRAEDTAVYYCAKEGTSSYRGWMDVWGQGTLVTVSS

SEQ ID NO: 124 - protein, 107 aa, synthetic construct
DIQMTQSPSSLSASVGDRVTITCRASQSISSYLNWYQQKPGKAPKLLIYAASRLQSGVPSRFSGSGSGTDFTLTISSLQPEDFATYYCQQSYSTPWTFGQGTKVEIK

SEQ ID NO: 125 - protein, 5 aa, synthetic construct
DYAMS

SEQ ID NO: 126 - protein, 17 aa, synthetic construct
RISQSGSYTYYADSVKG

SEQ ID NO: 127 - protein, 12 aa, synthetic construct
EGTSSYRGWMDV

SEQ ID NO: 128 - protein, 11 aa, synthetic construct
RASQSISNWLN

SEQ ID NO: 129 - protein, 7 aa, synthetic construct
ATSRLQS

SEQ ID NO: 130 - protein, 9 aa, synthetic construct
QQSYSTPWT

SEQ ID NO: 131 - protein, 30 aa, synthetic construct; identical to SEQ ID NO: 7

SEQ ID NO: 132 - protein, 14 aa, synthetic construct
WVRQAPGKGLEWVS

SEQ ID NO: 133 - protein, 32 aa, synthetic construct; identical to SEQ ID NO: 9

SEQ ID NO: 134 - protein, 11 aa, synthetic construct
WGQGTLVTVSS

SEQ ID NO: 135 - protein, 23 aa, synthetic construct
DIQMTQSPSSLSASVGDRVTITC

SEQ ID NO: 136 - protein, 15 aa, synthetic construct
WYQQKPGKAPKLLIY

SEQ ID NO: 137 - protein, 32 aa, synthetic construct; identical to SEQ ID NO: 29

SEQ ID NO: 138 - protein, 10 aa, synthetic construct
FGQGTKVEIK

SEQ ID NO: 139 - protein, 107 aa, synthetic construct
DIQMTQSPSSLSASVGDRVTITCRASQSISNWLNWYQQKPGKAPKLLIYATSRLQSGVPSRFSGSGSGTDFTLTISSLQPEDFATYYCQQSYSTPWTFGQGTKVEIK

SEQ ID NO: 140 - protein, 5 aa, synthetic construct
SYAMS

SEQ ID NO: 141 - protein, 17 aa, synthetic construct
RISGSGGYKYYADSVKG

SEQ ID NO: 142 - protein, 12 aa, synthetic construct
EGTSSYRGWMDV

SEQ ID NO: 143 - protein, 11 aa, synthetic construct
RASQSISNYLN

SEQ ID NO: 144 - protein, 7 aa, synthetic construct
ATSTLQS

SEQ ID NO: 145 - protein, 9 aa, synthetic construct
QQSYTTPWT

SEQ ID NO: 146 - protein, 30 aa, synthetic construct; identical to SEQ ID NO: 7

SEQ ID NO: 147 - protein, 14 aa, synthetic construct
WVRQAPGKGLEWVS

SEQ ID NO: 148 - protein, 32 aa, synthetic construct; identical to SEQ ID NO: 9

SEQ ID NO: 149 - protein, 11 aa, synthetic construct
WGQGTLVTVSS

SEQ ID NO: 150 - protein, 23 aa, synthetic construct
DIQMTQSPSSLSASVGDRVTITC

SEQ ID NO: 151 - protein, 15 aa, synthetic construct
WYQQKPGKAPKLLIY

SEQ ID NO: 152 - protein, 32 aa, synthetic construct; identical to SEQ ID NO: 29

SEQ ID NO: 153 - protein, 10 aa, synthetic construct
FGQGTKVEIK

SEQ ID NO: 154 - protein, 121 aa, synthetic construct
EVQLVESGGGLVQPGGSLRLSCAASGFTFSSYAMSWVRQAPGKGLEWVSRISGSGGYKYYADSVKGRFTISRDNSKNTLYLQMNSLRAEDTAVYYCAKEGTSSYRGWMDVWGQGTLVTVSS

SEQ ID NO: 155 - protein, 106 aa, synthetic construct
IQMTQSPSSLSASVGDRVTITCRASQSISNYLNWYQQKPGKAPKLLIYATSTLQSGVPSRFSGSGSGTDFTLTISSLQPEDFATYYCQQSYTTPWTFGQGTKVEIK

SEQ ID NO: 156 - protein, 5 aa, synthetic construct
DYAMS

SEQ ID NO: 157 - protein, 17 aa, synthetic construct
RISSSGSYTYYADSVKG

SEQ ID NO: 158 - protein, 12 aa, synthetic construct
EGTSKYRGWMDV

SEQ ID NO: 159 - protein, 11 aa, synthetic construct
RASQSISNYLN

SEQ ID NO: 160 - protein, 7 aa, synthetic construct
AASTLQS

SEQ ID NO: 161 - protein, 9 aa, synthetic construct
QQSYSTPWT

SEQ ID NO: 162 - protein, 30 aa, synthetic construct; identical to SEQ ID NO: 7

SEQ ID NO: 163 - protein, 14 aa, synthetic construct
WVRQAPGKGLEWVS

SEQ ID NO: 164 - protein, 32 aa, synthetic construct; identical to SEQ ID NO: 9

SEQ ID NO: 165 - protein, 11 aa, synthetic construct
WGQGTLVTVSS

SEQ ID NO: 166 - protein, 23 aa, synthetic construct
DIQMTQSPSSLSASVGDRVTITC

SEQ ID NO: 167 - protein, 15 aa, synthetic construct
WYQQKPGKAPKLLIY

SEQ ID NO: 168 - protein, 32 aa, synthetic construct; identical to SEQ ID NO: 29

SEQ ID NO: 169 - protein, 10 aa, synthetic construct
FGQGTKVEIK

SEQ ID NO: 170 - protein, 121 aa, synthetic construct
EVQLVESGGGLVQPGGSLRLSCAASGFTFSDYAMSWVRQAPGKGLEWVSRISSSGSYTYYADSVKGRFTISRDNSKNTLYLQMNSLRAEDTAVYYCAKEGTSKYRGWMDVWGQGTLVTVSS

SEQ ID NO: 171 - protein, 107 aa, synthetic construct
DIQMTQSPSSLSASVGDRVTITCRASQSISNYLNWYQQKPGKAPKLLIYAASTLQSGVPSRFSGSGSGTDFTLTISSLQPEDFATYYCQQSYSTPWTFGQGTKVEIK

SEQ ID NO: 172 - protein, 5 aa, synthetic construct
DYAMS

SEQ ID NO: 173 - protein, 17 aa, synthetic construct
RISGTGSYKYYADSVKG

SEQ ID NO: 174 - protein, 12 aa, synthetic construct
EGTSTYRGWMDV

SEQ ID NO: 175 - protein, 11 aa, synthetic construct
RASQSISNYLN

SEQ ID NO: 176 - protein, 7 aa, synthetic construct
ATSRLQS

SEQ ID NO: 177 - protein, 9 aa, synthetic construct
QQSYTTPWT

SEQ ID NO: 178 - protein, 30 aa, synthetic construct; identical to SEQ ID NO: 7

SEQ ID NO: 179 - protein, 14 aa, synthetic construct
WVRQAPGKGLEWVS

SEQ ID NO: 180 - protein, 32 aa, synthetic construct; identical to SEQ ID NO: 9

SEQ ID NO: 181 - protein, 11 aa, synthetic construct
WGQGTLVTVSS

SEQ ID NO: 182 - protein, 23 aa, synthetic construct
DIQMTQSPSSLSASVGDRVTITC

SEQ ID NO: 183 - protein, 15 aa, synthetic construct
WYQQKPGKAPKLLIY

SEQ ID NO: 184 - protein, 32 aa, synthetic construct; identical to SEQ ID NO: 29

SEQ ID NO: 185 - protein, 10 aa, synthetic construct
FGQGTKVEIK

SEQ ID NO: 186 - protein, 121 aa, synthetic construct
EVQLVESGGGLVQPGGSLRLSCAASGFTFSDYAMSWVRQAPGKGLEWVSRISGTGSYKYYADSVKGRFTISRDNSKNTLYLQMNSLRAEDTAVYYCAKEGTSTYRGWMDVWGQGTLVTVSS

SEQ ID NO: 187 - protein, 107 aa, synthetic construct
DIQMTQSPSSLSASVGDRVTITCRASQSISNYLNWYQQKPGKAPKLLIYATSRLQSGVPSRFSGSGSGTDFTLTISSLQPEDFATYYCQQSYTTPWTFGQGTKVEIK

SEQ ID NO: 188 - protein, 5 aa, synthetic construct
SYAMS

SEQ ID NO: 189 - protein, 17 aa, synthetic construct
RISGSGSYTYYADSVKG

SEQ ID NO: 190 - protein, 12 aa, synthetic construct
EGASSYRGWMDV

SEQ ID NO: 191 - protein, 10 aa, synthetic construct
ASQSISNYLN

SEQ ID NO: 192 - protein, 7 aa, synthetic construct
ATSRLQS

SEQ ID NO: 193 - protein, 9 aa, synthetic construct
QQSHSTPWT

SEQ ID NO: 194 - protein, 30 aa, synthetic construct; identical to SEQ ID NO: 7

SEQ ID NO: 195 - protein, 14 aa, synthetic construct
WVRQAPGKGLEWVS

SEQ ID NO: 196 - protein, 32 aa, synthetic construct; identical to SEQ ID NO: 9

SEQ ID NO: 197 - protein, 11 aa, synthetic construct
WGQGTLVTVSS

SEQ ID NO: 198 - protein, 24 aa, synthetic construct
DIQMTQSPSSLSASVGDRVTITCR

SEQ ID NO: 199 - protein, 15 aa, synthetic construct
WYQQKPGKAPKLLIY

SEQ ID NO: 200 - protein, 32 aa, synthetic construct; identical to SEQ ID NO: 29

SEQ ID NO: 201 - protein, 10 aa, synthetic construct
FGQGTKVEIK

SEQ ID NO: 202 - protein, 121 aa, synthetic construct
EVQLVESGGGLVQPGGSLRLSCAASGFTFSSYAMSWVRQAPGKGLEWVSRISGSGSYTYYADSVKGRFTISRDNSKNTLYLQMNSLRAEDTAVYYCAKEGASSYRGWMDVWGQGTLVTVSS

SEQ ID NO: 203 - protein, 107 aa, synthetic construct
DIQMTQSPSSLSASVGDRVTITCRASQSISNYLNWYQQKPGKAPKLLIYATSRLQSGVPSRFSGSGSGTDFTLTISSLQPEDFATYYCQQSHSTPWTFGQGTKVEIK

SEQ ID NO: 204 - protein, 7 aa, synthetic construct
SSSTYWS

SEQ ID NO: 205 - protein, 16 aa, synthetic construct
GIAYSGSTYYNPSLKS

SEQ ID NO: 206 - protein, 10 aa, synthetic construct
GVRRAVPEDY

SEQ ID NO: 207 - protein, 9 aa, synthetic construct
QAVSSNYLA

SEQ ID NO: 208 - protein, 7 aa, synthetic construct
GASSRAT

SEQ ID NO: 209 - protein, 9 aa, synthetic construct
QQVVHSPYT

SEQ ID NO: 210 - protein, 30 aa, synthetic construct
QLQLQESGPGLVKPSETLSLTCTVSGGSIS

SEQ ID NO: 211 - protein, 14 aa, synthetic construct
WIRQPPGKGLEWIG

SEQ ID NO: 212 - protein, 32 aa, synthetic construct
RVTISVDTSKNQFSLKLSSVTAADTAVYYCAR

SEQ ID NO: 213 - protein, 11 aa, synthetic construct
WGQGTLVTVSS

SEQ ID NO: 214 - protein, 26 aa, synthetic construct
EIVLTQSPGTLSLSPGERATLSCQAS

SEQ ID NO: 215 - protein, 15 aa, synthetic construct
WYQQKPGQAPRLLIY

SEQ ID NO: 216 - protein, 32 aa, synthetic construct
GIPDRFSGSGSGTDFTLTISRLEPEDFAVYYC

SEQ ID NO: 217 - protein, 10 aa, synthetic construct
FGGGTKVEIK

SEQ ID NO: 218 - protein, 120 aa, synthetic construct
QLQLQESGPGLVKPSETLSLTCTVSGGSISSSSTYWSWIRQPPGKGLEWIGGIAYSGSTYYNPSLKSRVTISVDTSKNQFSLKLSSVTAADTAVYYCARGVRRAVPEDYWGQGTLVTVSS

SEQ ID NO: 219 - protein, 108 aa, synthetic construct
EIVLTQSPGTLSLSPGERATLSCQASQAVSSNYLAWYQQKPGQAPRLLIYGASSRATGIPDRFSGSGSGTDFTLTISRLEPEDFAVYYCQQVVHSPYTFGGGTKVEIK

SEQ ID NO: 220 - protein, 330 aa, synthetic construct [sequence omitted]

SEQ ID NO: 221 - protein, 107 aa, synthetic construct [sequence omitted]

SEQ ID NO: 222 - protein, 604 aa, synthetic construct
ASTKGPSVFPLAPSSKSTSGGTAALGCLVKDYFPEPVTVSWNSGALTSGVHTFPAVLQSSGLYSLSSVVTVPSSSLGTQTYICNVNHKPSNTKVDKKVEPKSCRNTGRGGEEKKKEKEKEEQEERETKTPECPSHTQPLGVDKTHTCPPCPAPELLGGPSVFLFPPKPKDTLMISRTPEVTCVVVDVSHEDPEVKFNWYVDGVEVHNAKTKPREEQYNSTYRVVSVLTVLHQDWLNGKEYKCKVSNKALPAPIEKTISKAKGQPREPQVYTLPPSRDELTKNQVSLTCLVKGFYPSDIAVEWESNGQPENNYKTTPPVLDSDGSFFLYSKLTVDKSRWQQGNVFSCSVMHEALHNHYTQKSLSLSPGKQDTAIRVFAIPPSFASIFLTKSTKLTCLVTDLTTYDSVTISWTRQNGEAVKTHTNISESHPNATFSAVGEASICEDDWNSGERFTCTVTHTDLPSPLKQTISRPKGVALHRPDVYLLPPAREQLNSRESATITCLVTGFSPADVFVQWMQRGQPLSPEKYVTSAPMPEPQAPGRYFAHSILTVSEEEWNTGETYTCVVAHEALPNRVTERTVDKSTGKPTLYNVSLVMSDTAGTCY

SEQ ID NO: 223 - protein, 137 aa, synthetic construct
QEDERIVLVDNKCKCARITSRIIRSSEDPNEDIVERNIRIIVPLNNRENISDPTSPLRTRFVYHLSDLCKKCDPTEVELDNQIVTATQSNICDEDSATETCYTYDWNKCYTAVVPLVYGGETKMVETALTPDACYPD